European Patent Specification EP 3 701 022 B1, published March 1, 2023. Title: BETA-LACTAMASE VARIANTS. Applicant: DA VOLTERRA et al. The sequence listing filed with the application follows.

SEQUENCE LISTING (23 sequences)

SEQ ID NO: 1 - protein, 240 aa, artificial
  wild-type VIM-2
VDSSGEYPTVSEIPVGEVRLYQIADGVWSHIATQSFDGAVYPSNGLIVRDGDELLLIDTAWGAKNTAALLAEIEKQIGLPVTRAVSTHFHDDRVGGVDVLRAAGVATYASPSTRRLAEVEGNEIPTHSLEGLSSSGDAVRFGPVELFYPGAAHSTDNLVVYVPSASVLYGGCAIYELSRTSAGNVADADLAEWPTSIERIQQHYPEAQFVIPGHGLPGGLDLLKHTTNVVKAHTNRSVVE

SEQ ID NO: 2 - protein, 26 aa, artificial
  VIM-2 signal peptide
MFKLLSKLLVYLTASIMAIASPLAFS

SEQ ID NO: 3 - protein, 240 aa, artificial
  VIM-2 variant
VDSSGEYPTASEIPVGEVRLYQIADGVWSHIATQSFDGAVYPSNGLIVRDGDELLLIDTAWGAKNTAALLAEIEKQIGLPVTRAVSTHFHDDRVGGVDVLRAAGVATYASPSTRRLAEVEGNEIPTHSLEGLSSSGDAVRFGPVELFYPGAAHSTDNLVVYVPSASVLYGGCAIYELSRTSAGNVADADLAEWPTSIERIQQHYPEAQFVIPGHGLPGGLDLLKHTTNVVKAHTNRSVVE

SEQ ID NO: 4 - protein, 240 aa, artificial
  VIM-2 variant
VDSSGEYPTASEIPVGEVRLYHIADGVWSHIATRSFDGAVYPSNGLIVRDGDELLLIDTAWGAKNTAALLAEIEKQIGLPVTRAVSTHFHDDRVGGVDVLRAAGVATYASPSTRRLAEVEGNEIPTHSLEGLSSSGDAVRFGPVELFYPGAAHSTDNLVVYVPSASVLYGGCAIYELSRTSAGNVADADLAEWPTSIERIQQHYPEAQFVIPGHGLPGGLDLLKHTTNVVKAHTNRSVVE

SEQ ID NO: 5 - protein, 240 aa, artificial
  VIM-2 variant
VDSSGEYPTASEIPVGEVRLYNIADGVWSHIATRSFDGAVYPSNGLIVRDGDELLLIDTAWGAKNTAALLAEIEKQIGLPVTRAVSTHFHDDRVGGVDVLRAAGVATYASPSTRRLAEVEGNEIPTHSLEGLSSSGDAVRFGPVELFYPGAAHSTDNLVVYVPSASVLYGGCAIYELSRTSAGNVADADLAEWPTSIERIQQHYPEAQFVIPGHGLPGGLDLLKHTTNVVKAHTNRSVVE

SEQ ID NO: 6 - protein, 240 aa, artificial
  VIM-2 variant
VDSSGEYPTASEIPVGEVRLYQIADGVWSHIATRSFDGAVYPSNGLIVRDGDELLLIDTAWGAKNTAALLAEIEKQIGLPVTRAVSTHFHDDRVGGVDVLRAAGVATYASPSTRRLAEVEGNEIPTHSLDGLSSSGDAVRFGPVELFYPGAAHSTDNLVVYVPSASVLYGGCAIYELSRTSAGNVADADLAEWPTSIERIQQHYPEAQFVIPGHGLPGGLDLLKHTTNVVKAHTNRSVVE

SEQ ID NO: 7 - protein, 240 aa, artificial
  VIM-2 variant
VDSSGEYPTASEIPVGEVRLYNIADGVWSHIATRSFDGAVYPSNGLIVRDGDELLLIDTAWGAKNTAALLAEIEKQIGLPVTRAVSTHFHDDRVGGVDVLRAAGVATYASPSTRRLAEVEGNEIPTHSLDGLSSSGDAVRFGPVELFYPGAAHSTDNLVVYVPSASVLYGGCAIYELSRTSAGNVADADLAEWPTSIERIQQHYPEAQFVIPGHGLPGGLDLLKHTTNVVKAHTNRSVVE

SEQ ID NO: 8 - protein, 240 aa, artificial
  VIM-2 variant
VDSSGEYPTASEIPVGEVRLYHIADGVWSHIATRSFDGAVYPSNGLIVRDGDELLLIDTAWGAKNTAALLAEIEKQIGLPVTRAVSTHFHDDRVGGVDVLRAAGVATYASPSTRRLAEVEGNEIPTHSLDGLSSSGDAVRFGPVELFYPGAAHSTDNLVVYVPSASVLYGGCAIYELSRTSAGNVADADLAEWPTSIERIQQHYPEAQFVIPGHGLPGGLDLLKHTTNVVKAHTNRSVVE

SEQ ID NO: 9 - protein, 235 aa, artificial
  VIM-2 variant
VDSSGEYPTASEIPVGEVRLYHIADGVWSHIATRSFDGAVYPSNGLIVRDGDELLLIDTAWGAKNTAALLAEIEKQIGLPVTRAVSTHFHDDRVGGVDVLRAAGVATYASPSTRRLAEVEGNEIPTHSLEGLSSSGDAVRFGPVELFYPGAAHSTDNLVVYVPSASVLYGGCAIYELSRTSAGNVADADLAEWPTSIERIQQHYPEAQFVIPGHGLPGGLDLLKHTTNVVKAHTN

SEQ ID NO: 10 - protein, 235 aa, artificial
  VIM-2 variant
VDSSGEYPTASEIPVGEVRLYNIADGVWSHIATRSFDGAVYPSNGLIVRDGDELLLIDTAWGAKNTAALLAEIEKQIGLPVTRAVSTHFHDDRVGGVDVLRAAGVATYASPSTRRLAEVEGNEIPTHSLEGLSSSGDAVRFGPVELFYPGAAHSTDNLVVYVPSASVLYGGCAIYELSRTSAGNVADADLAEWPTSIERIQQHYPEAQFVIPGHGLPGGLDLLKHTTNVVKAHTN

SEQ ID NO: 11 - protein, 235 aa, artificial
  VIM-2 variant
VDSSGEYPTASEIPVGEVRLYQIADGVWSHIATRSFDGAVYPSNGLIVRDGDELLLIDTAWGAKNTAALLAEIEKQIGLPVTRAVSTHFHDDRVGGVDVLRAAGVATYASPSTRRLAEVEGNEIPTHSLDGLSSSGDAVRFGPVELFYPGAAHSTDNLVVYVPSASVLYGGCAIYELSRTSAGNVADADLAEWPTSIERIQQHYPEAQFVIPGHGLPGGLDLLKHTTNVVKAHTN

SEQ ID NO: 12 - protein, 235 aa, artificial
  VIM-2 variant
VDSSGEYPTASEIPVGEVRLYNIADGVWSHIATRSFDGAVYPSNGLIVRDGDELLLIDTAWGAKNTAALLAEIEKQIGLPVTRAVSTHFHDDRVGGVDVLRAAGVATYASPSTRRLAEVEGNEIPTHSLDGLSSSGDAVRFGPVELFYPGAAHSTDNLVVYVPSASVLYGGCAIYELSRTSAGNVADADLAEWPTSIERIQQHYPEAQFVIPGHGLPGGLDLLKHTTNVVKAHTN

SEQ ID NO: 13 - protein, 235 aa, artificial
  VIM-2 variant
VDSSGEYPTASEIPVGEVRLYHIADGVWSHIATRSFDGAVYPSNGLIVRDGDELLLIDTAWGAKNTAALLAEIEKQIGLPVTRAVSTHFHDDRVGGVDVLRAAGVATYASPSTRRLAEVEGNEIPTHSLDGLSSSGDAVRFGPVELFYPGAAHSTDNLVVYVPSASVLYGGCAIYELSRTSAGNVADADLAEWPTSIERIQQHYPEAQFVIPGHGLPGGLDLLKHTTNVVKAHTN

SEQ ID NO: 14 - protein, 240 aa, artificial
  VIM-2 variant
MDSSGEYPTASEIPVGEVRLYHIADGVWSHIATRSFDGAVYPSNGLIVRDGDELLLIDTAWGAKNTAALLAEIEKQIGLPVTRAVSTHFHDDRVGGVDVLRAAGVATYASPSTRRLAEVEGNEIPTHSLEGLSSSGDAVRFGPVELFYPGAAHSTDNLVVYVPSASVLYGGCAIYELSRTSAGNVADADLAEWPTSIERIQQHYPEAQFVIPGHGLPGGLDLLKHTTNVVKAHTNRSVVE

SEQ ID NO: 15 - protein, 240 aa, artificial
  VIM-2 variant
MDSSGEYPTASEIPVGEVRLYNIADGVWSHIATRSFDGAVYPSNGLIVRDGDELLLIDTAWGAKNTAALLAEIEKQIGLPVTRAVSTHFHDDRVGGVDVLRAAGVATYASPSTRRLAEVEGNEIPTHSLEGLSSSGDAVRFGPVELFYPGAAHSTDNLVVYVPSASVLYGGCAIYELSRTSAGNVADADLAEWPTSIERIQQHYPEAQFVIPGHGLPGGLDLLKHTTNVVKAHTNRSVVE

SEQ ID NO: 16 - protein, 240 aa, artificial
  VIM-2 variant
MDSSGEYPTASEIPVGEVRLYQIADGVWSHIATRSFDGAVYPSNGLIVRDGDELLLIDTAWGAKNTAALLAEIEKQIGLPVTRAVSTHFHDDRVGGVDVLRAAGVATYASPSTRRLAEVEGNEIPTHSLDGLSSSGDAVRFGPVELFYPGAAHSTDNLVVYVPSASVLYGGCAIYELSRTSAGNVADADLAEWPTSIERIQQHYPEAQFVIPGHGLPGGLDLLKHTTNVVKAHTNRSVVE

SEQ ID NO: 17 - protein, 240 aa, artificial
  VIM-2 variant
MDSSGEYPTASEIPVGEVRLYNIADGVWSHIATRSFDGAVYPSNGLIVRDGDELLLIDTAWGAKNTAALLAEIEKQIGLPVTRAVSTHFHDDRVGGVDVLRAAGVATYASPSTRRLAEVEGNEIPTHSLDGLSSSGDAVRFGPVELFYPGAAHSTDNLVVYVPSASVLYGGCAIYELSRTSAGNVADADLAEWPTSIERIQQHYPEAQFVIPGHGLPGGLDLLKHTTNVVKAHTNRSVVE

SEQ ID NO: 18 - protein, 240 aa, artificial
  VIM-2 variant
MDSSGEYPTASEIPVGEVRLYHIADGVWSHIATRSFDGAVYPSNGLIVRDGDELLLIDTAWGAKNTAALLAEIEKQIGLPVTRAVSTHFHDDRVGGVDVLRAAGVATYASPSTRRLAEVEGNEIPTHSLDGLSSSGDAVRFGPVELFYPGAAHSTDNLVVYVPSASVLYGGCAIYELSRTSAGNVADADLAEWPTSIERIQQHYPEAQFVIPGHGLPGGLDLLKHTTNVVKAHTNRSVVE

SEQ ID NO: 19 - protein, 235 aa, artificial
  VIM-2 variant
MDSSGEYPTASEIPVGEVRLYHIADGVWSHIATRSFDGAVYPSNGLIVRDGDELLLIDTAWGAKNTAALLAEIEKQIGLPVTRAVSTHFHDDRVGGVDVLRAAGVATYASPSTRRLAEVEGNEIPTHSLEGLSSSGDAVRFGPVELFYPGAAHSTDNLVVYVPSASVLYGGCAIYELSRTSAGNVADADLAEWPTSIERIQQHYPEAQFVIPGHGLPGGLDLLKHTTNVVKAHTN

SEQ ID NO: 20 - protein, 235 aa, artificial
  VIM-2 variant
MDSSGEYPTASEIPVGEVRLYNIADGVWSHIATRSFDGAVYPSNGLIVRDGDELLLIDTAWGAKNTAALLAEIEKQIGLPVTRAVSTHFHDDRVGGVDVLRAAGVATYASPSTRRLAEVEGNEIPTHSLEGLSSSGDAVRFGPVELFYPGAAHSTDNLVVYVPSASVLYGGCAIYELSRTSAGNVADADLAEWPTSIERIQQHYPEAQFVIPGHGLPGGLDLLKHTTNVVKAHTN

SEQ ID NO: 21 - protein, 235 aa, artificial
  VIM-2 variant
MDSSGEYPTASEIPVGEVRLYQIADGVWSHIATRSFDGAVYPSNGLIVRDGDELLLIDTAWGAKNTAALLAEIEKQIGLPVTRAVSTHFHDDRVGGVDVLRAAGVATYASPSTRRLAEVEGNEIPTHSLDGLSSSGDAVRFGPVELFYPGAAHSTDNLVVYVPSASVLYGGCAIYELSRTSAGNVADADLAEWPTSIERIQQHYPEAQFVIPGHGLPGGLDLLKHTTNVVKAHTN

SEQ ID NO: 22 - protein, 235 aa, artificial
  VIM-2 variant
MDSSGEYPTASEIPVGEVRLYNIADGVWSHIATRSFDGAVYPSNGLIVRDGDELLLIDTAWGAKNTAALLAEIEKQIGLPVTRAVSTHFHDDRVGGVDVLRAAGVATYASPSTRRLAEVEGNEIPTHSLDGLSSSGDAVRFGPVELFYPGAAHSTDNLVVYVPSASVLYGGCAIYELSRTSAGNVADADLAEWPTSIERIQQHYPEAQFVIPGHGLPGGLDLLKHTTNVVKAHTN

SEQ ID NO: 23 - protein, 235 aa, artificial
  VIM-2 variant
MDSSGEYPTASEIPVGEVRLYHIADGVWSHIATRSFDGAVYPSNGLIVRDGDELLLIDTAWGAKNTAALLAEIEKQIGLPVTRAVSTHFHDDRVGGVDVLRAAGVATYASPSTRRLAEVEGNEIPTHSLDGLSSSGDAVRFGPVELFYPGAAHSTDNLVVYVPSASVLYGGCAIYELSRTSAGNVADADLAEWPTSIERIQQHYPEAQFVIPGHGLPGGLDLLKHTTNVVKAHTN